European Patent Application EP 4 144 863 A1, published March 8, 2023. Title: Method for detection of RNA virus. Applicant: TAKARA BIO INC. The sequence listing filed with the application follows.

SEQUENCE LISTING (13 sequences)

SEQ ID NO: 1 - DNA, 20 bp, Artificial Sequence
  PCR Forward Primer NIID_2019-nCOV_N_F2
aaattttggggaccaggaac

SEQ ID NO: 2 - DNA, 20 bp, Artificial Sequence
  PCR Reverse Primer NIID_2019-nCOV_N_R2
tggcagctgtgtaggtcaac

SEQ ID NO: 3 - DNA, 20 bp, Artificial Sequence
  Probe NIID_2019-nCOV_N_P2. 5'-end is labeled FAM and 3'-end is labeled BHQ1
atgtcgcgcattggcatgga

SEQ ID NO: 4 - RNA, 337 nt, Artificial Sequence
  RNA positive control sequence for 2019-nCoV N2 set
gggcagacgugguccagaacaaacccaaggaaauuuuggggaccaggaacuaaucagacggauccagcuagcgcauuggaucucgcaaauugcacaauuugcccccagcgcuucagcguucuucggaaugucgcgcauuggcauggaagucacaccuucgggaacgugguugaccuacacagcugccaucaaauuggaugacaaagauccaaauuucaaagaucaagucauuuugcugaauaagcauauugacgcauacaaaacauucccaccaacagagccuaaaaaggacaaaaagaagaaggcugaugaaacucaagccuuaccgcagagacag

SEQ ID NO: 5 - DNA, 29 bp, Artificial Sequence
  PCR Forward Primer IAmg-F01
ccmaggtcgaaacgtaygttctctctatc

SEQ ID NO: 6 - DNA, 32 bp, Artificial Sequence
  PCR Reverse Primer IAmg-R01
tgacagratyggtcttgtctttagccaytcca

SEQ ID NO: 7 - DNA, 22 bp, Artificial Sequence
  Probe IAmg-PB1. 5'-end is labeled FAM and 3'-end is labeled BHQ1
atytcggctttgagggggcctg

SEQ ID NO: 8 - DNA, 23 bp, Artificial Sequence
  PCR Forward Primer N1_SARS COV_F
gaccccaatcaaaccaacgtagt

SEQ ID NO: 9 - DNA, 24 bp, Artificial Sequence
  PCR Reverse Primer N1_SARS COV_R
tctggttattgtcagttgaatctg

SEQ ID NO: 10 - DNA, 24 bp, Artificial Sequence
  N1_SARS COV_P. 5'-end is labeled Cy5 and 3'-end is labeled BHQ3
cccccgcattacatttggtggacc

SEQ ID NO: 11 - DNA, 20 bp, Artificial Sequence
  PCR Forward Primer N2_SARS COV_F
ttacaaacattggccgcaaa

SEQ ID NO: 12 - DNA, 18 bp, Artificial Sequence
  PCR Reverse Primer N2_SARS COV_R
gcgtgacattccaaagaa

SEQ ID NO: 13 - DNA, 23 bp, Artificial Sequence
  N2_SARS COV_P. 5'-end is labeled Cy5 and 3'-end is labeled BHQ3
acaatttgctccaagtgcctctg